European Patent Application EP 4 600 368 A1, published August 13, 2025. Title: A METHOD FOR AN ENZYMATICALLY PRODUCTION OF AN AMIDE COMPOUND. Applicant: ADISSEO FRANCE S.A.S. The sequence listing filed with the application follows.

SEQUENCE LISTING (4 sequences)

SEQ ID NO: 1 - protein, 205 aa, Pseudonocardia thermophila
MTENILRKSDEEIQKEITARVKALESMLIEQGILTTSMIDRMAEIYENEVGPHLGAKVVVKAWTDPEFKKRLLADGTEACKELGIGGLQGEDMMWVENTDEVHHVVVCTLCSCYPWPVLGLPPNWFKEPQYRSRVVREPRQLLKEEFGFEVPPSKEIKVWDSSSEMRFVVLPQRPAGTDGWSEEELATLVTRESMIGVEPAKAVA

SEQ ID NO: 2 - protein, 233 aa, Pseudonocardia thermophila
MNGVYDVGGTDGLGPINRPADEPVFRAEWEKVAFAMFPATFRAGFMGLDEFRFGIEQMNPAEYLESPYYWHWIRTYIHHGVRTGKIDLEELERRTQYYRENPDAPLPEHEQKPELIEFVNQAVYGGLPASREVDRPPKFKEGDVVRFSTASPKGHARRARYVRGKTGTVVKHHGAYIYPDTAGNGLGECPEHLYTVRFTAQELWGPEGDPNSSVYYDCWEPYIELVDTKAAAA

SEQ ID NO: 3 - DNA, 618 bp, Pseudonocardia thermophila
  source 1..618: mol_type = genomic DNA
atgaccgagaacatcctgcgcaagtcggacgaggagatccagaaggagatcacggcgcgggtcaaggccctggagtcgatgctcatcgaacagggcatcctcaccacgtcgatgatcgaccggatggccgagatctacgagaacgaggtcggcccgcacctcggcgcgaaggtcgtcgtgaaggcctggaccgacccggagttcaagaagcgtctgctcgccgacggcaccgaggcctgcaaggagctcggcatcggcggcctgcagggcgaggacatgatgtgggtggagaacaccgacgaggtccaccacgtcgtcgtgtgcacgctctgctcctgctacccgtggccggtgctggggctgccgccgaactggttcaaggagccgcagtaccgctcccgcgtggtgcgtgagccccggcagctgctcaaggaggagttcggcttcgaggtcccgccgagcaaggagatcaaggtctgggactccagctccgagatgcgcttcgtcgtcctcccgcagcgccccgcgggcaccgacgggtggagcgaggaggagctcgccaccctcgtcacccgcgagtcgatgatcggcgtcgaaccggcgaaggcggtcgcgtga

SEQ ID NO: 4 - DNA, 702 bp, Pseudonocardia thermophila
  source 1..702: mol_type = genomic DNA
atgaacggcgtgtacgacgtcggcggcaccgatgggctgggcccgatcaaccggcccgcggacgaaccggtcttccgcgccgagtgggagaaggtcgcgttcgcgatgttcccggcgacgttccgggccggcttcatgggcctggacgagttccggttcggcatcgagcagatgaacccggccgagtacctcgagtcgccgtactactggcactggatccgcacctacatccaccacggcgtccgcaccggcaagatcgatctcgaggagctggagcgccgcacgcagtactaccgggagaaccccgacgccccgctgcccgagcacgagcagaagccggagttgatcgagttcgtcaaccaggccgtctacggcgggctgcccgcaagccgggaggtcgaccgaccgcccaagttcaaggagggcgacgtggtgcggttctccaccgcgagcccgaagggccacgcccggcgcgcgcggtacgtgcgcggcaagaccgggacggtggtcaagcaccacggcgcgtacatctacccggacaccgccggcaacggcctgggcgagtgccccgagcacctctacaccgtccgcttcacggcccaggagctgtgggggccggaaggggacccgaactccagcgtctactacgactgctgggagccctacatcgagctcgtcgacacgaaggcggccgcggcatga